European Patent Application EP 4 173 641 A1, published May 3, 2023. Title: Pharmaceutical composition for retinal neurodegenerative disease comprising inhibitor of Prox1 as an active ingredient. Applicant: Korea Advanced Institute of Science and Technology. The sequence listing filed with the application follows.

SEQUENCE LISTING (4 sequences)

SEQ ID NO: 1 - DNA, 2214 bp, Homo sapiens_Prox1
atgcctgaccatgacagcacagccctcttaagccggcaaaccaagaggagaagagttgacattggagtgaaaaggacggtagggacagcatctgcattttttgctaaggcaagagcaacgttttttagtgccatgaatccccaaggttctgagcaggatgttgagtattcagtggtgcagcatgcagatggggaaaagtcaaatgtactccgcaagctgctgaagagggcgaactcgtatgaagatgccatgatgccttttccaggagcaaccataatttcccagctgttgaaaaataacatgaacaaaaatggtggcacggagcccagtttccaagccagcggtctctctagtacaggctccgaagtacatcaggaggatatatgcagcaactcttcaagagacagccccccagagtgtctttccccttttggcaggcctactatgagccagtttgatatggatcgcttatgtgatgagcacctgagagcaaagcgcgcccgggttgagaatataattcggggtatgagccattcccccagtgtggcattaaggggcaatgaaaatgaaagagagatggccccgcagtctgtgagtccccgagaaagttacagagaaaacaaacgcaagcaaaagcttccccagcagcagcaacagagtttccagcagctggtttcagcccgaaaagaacagaagcgagaggagcgccgacagctgaaacagcagctggaggacatgcagaaacagctgcgccagctgcaggaaaagttctaccaaatctatgacagcactgattcggaaaatgatgaagatggtaacctgtctgaagacagcatgcgctcggagatcctggatgccagggcccaggactctgtcggaaggtcagataatgagatgtgcgagctagacccaggacagtttattgaccgagctcgagccctgatcagagagcaggaaatggctgaaaacaagccgaagcgagaaggcaacaacaaagaaagagaccatgggccaaactccttacaaccggaaggcaaacatttggctgagaccttgaaacaggaactgaacactgccatgtcgcaagttgtggacactgtggtcaaagtcttttcggccaagccctcccgccaggttcctcaggtcttcccacctctccagatcccccaggccagatttgcagtcaatggggaaaaccacaatttccacaccgccaaccagcgcctgcagtgctttggcgacgtcatcattccgaaccccctggacacctttggcaatgtgcagatggccagttccactgaccagacagaagcactgcccctggttgtccgcaaaaactcctctgaccagtctgcctccggccctgccgctggcggccaccaccagcccctgcaccagtcgcctctctctgccaccacgggcttcaccacgtccaccttccgccaccccttcccccttcccttgatggcctatccatttcagagcccattaggtgctccctccggctccttctctggaaaagacagagcctctcctgaatccttagacttaactagggataccacgagtctgaggaccaagatgtcatctcaccacctgagccaccacccttgttcaccagcacacccgcccagcaccgccgaagggctctccttgtcgctcataaagtccgagtgcggcgatcttcaagatatgtctgaaatatcaccttattcgggaagtgcaatgcaggaaggattgtcacccaatcacttgaaaaaagcaaagctcatgtttttttatacccgttatcccagctccaatatgctgaagacctacttctccgacgtaaagttcaacagatgcattacctctcagctcatcaagtggtttagcaatttccgtgagttttactacattcagatggagaagtacgcacgtcaagccatcaacgatggggtcaccagtactgaagagctgtctataaccagagactgtgagctgtacagggctctgaacatgcactacaataaagcaaatgactttgaggttccagagagattcctggaagttgctcagatcacattacgggagtttttcaatgccattatcgcaggcaaagatgttgatccttcctggaagaaggccatatacaaggtcatctgcaagctggatagtgaagtccctgagattttcaaatccccgaactgcctacaagagctgcttcatgagtag

SEQ ID NO: 2 - protein, 737 aa, Homo sapiens_Prox1
MPDHDSTALLSRQTKRRRVDIGVKRTVGTASAFFAKARATFFSAMNPQGSEQDVEYSVVQHADGEKSNVLRKLLKRANSYEDAMMPFPGATIISQLLKNNMNKNGGTEPSFQASGLSSTGSEVHQEDICSNSSRDSPPECLSPFGRPTMSQFDMDRLCDEHLRAKRARVENIIRGMSHSPSVALRGNENEREMAPQSVSPRESYRENKRKQKLPQQQQQSFQQLVSARKEQKREERRQLKQQLEDMQKQLRQLQEKFYQIYDSTDSENDEDGNLSEDSMRSEILDARAQDSVGRSDNEMCELDPGQFIDRARALIREQEMAENKPKREGNNKERDHGPNSLQPEGKHLAETLKQELNTAMSQVVDTVVKVFSAKPSRQVPQVFPPLQIPQARFAVNGENHNFHTANQRLQCFGDVIIPNPLDTFGNVQMASSTDQTEALPLVVRKNSSDQSASGPAAGGHHQPLHQSPLSATTGFTTSTFRHPFPLPLMAYPFQSPLGAPSGSFSGKDRASPESLDLTRDTTSLRTKMSSHHLSHHPCSPAHPPSTAEGLSLSLIKSECGDLQDMSEISPYSGSAMQEGLSPNHLKKAKLMFFYTRYPSSNMLKTYFSDVKFNRCITSQLIKWFSNFREFYYIQMEKYARQAINDGVTSTEELSITRDCELYRALNMHYNKANDFEVPERFLEVAQITLREFFNAIIAGKDVDPSWKKAIYKVICKLDSEVPEIFKSPNCLQELLHE

SEQ ID NO: 3 - DNA, 2214 bp, Mus musculus_Prox1
atgcctgaccatgacagcacagccctcttaagccggcaaaccaagaggagaagggttgacattggagtgaaaaggacggtagggacagcatctgcattttttgctaaggcaagggcaacatttttcagtgccatgaatccccaaggttcagagcaggatgttgaatattctgtggtgcaacacgcagatggggaaaagtcgaacgtactccgcaagctgctgaagagggcgaactcgtatgaagatgccatgatgccttttccaggagcaactataatttcccagctgttgaaaaataacatgaacaaaaacggtggcaccgagcccagtttccaagccagcggactctctagcacaggctccgaagtacatcaggaggatatatgtagcaactcttcaagagacagccccccagagtgtctttccccttttggcaggcctactatgagccagtttgatgtggatcgcttatgtgatgagcacctgagagcaaagcgggcccgggttgagaatatcattcggggtatgagccattcccccagtgtggcattaaggggcaatgaaaatgaaagagagatggccccgcagtctgtgagtccccgagaaagttacagagaaaacaaacgcaagcagaagctgccccagcagcagcaacagagtttccagcagctggtttcagcccgaaaagaacagaagcgagaggagcgccgacagctgaaacagcagctggaagacatgcagaagcagctgcgccagctgcaggagaagttctaccaggtctatgacagcacagactccgaaaatgatgaagatggcgacctgtctgaagacagcatgcgctcggagatcctggatgcacgggcccaggactcggtggggcgctcagacaatgagatgtgtgagctggacccagggcagttcatcgacagggcccgagccctaatcagggagcaggagatggctgagaacaagcctaagcgagaaggcagcaacaaagaaagagaccacgggccaaactccttgcagccagaaggcaagcatctggcagagaccttaaaacaggagctgaacacggccatgtcgcaggtcgtggacacggtggtcaaagtcttctcagccaaaccctctcgccaggttcctcaggtcttcccacctctccagatcccccaggccagattcgcagtcaacggggaaaaccacaatttccacacggccaaccagcgcctgcaatgctttggtgatgtcatcattccgaaccccttggacacctttggcagtgtgcagatgcctagttccacagaccagacggaagcccttcccctggtggtccgaaaaaactcatccgagcaatctgcctctggcccggccactggcggccaccaccagcccctgcaccagtcacccctctccgccactgcaggcttcaccacccctagcttccgccatccctttcccctgcccttgatggcttatccatttcagagtccactaggtgctccctccggctccttctcggggaaggacagagcctctcctgagtccttagacttgactcgggacacaacaagtctgaggaccaagatgtcatcacaccatctgagccaccacccctgttcaccagcacacccacccagcaccgcagaaggactctctttgtcactcataaagtctgagtgtggagatcttcaagatatgtccgacatctcaccttattcaggaagcgcaatgcaggaagggctatcacccaatcacttgaaaaaggcaaaactcatgttcttttacacccgctaccccagctccaacatgctgaagacctacttctcggacgtgaagttcaacagatgcattacctcgcagctcatcaagtggttcagcaatttccgtgagttttactatatccagatggagaagtatgcgcgtcaagccatcaatgatggagtcaccagtacagaagagctctccatcaccagggattgtgaactataccgagccctcaacatgcactacaacaaagcaaatgactttgaggttccagagagattcctggaagttgcgcagatcacgttacgggagtttttcaatgccatcatcgcgggcaaagatgttgatccttcctggaagaaggccatttacaaggtcatctgcaagctggatagtgaagttcctgagattttcaaatcccctaactgcctacaagaactccttcacgagtag

SEQ ID NO: 4 - protein, 737 aa, Mus musculus_Prox1
MPDHDSTALLSRQTKRRRVDIGVKRTVGTASAFFAKARATFFSAMNPQGSEQDVEYSVVQHADGEKSNVLRKLLKRANSYEDAMMPFPGATIISQLLKNNMNKNGGTEPSFQASGLSSTGSEVHQEDICSNSSRDSPPECLSPFGRPTMSQFDVDRLCDEHLRAKRARVENIIRGMSHSPSVALRGNENEREMAPQSVSPRESYRENKRKQKLPQQQQQSFQQLVSARKEQKREERRQLKQQLEDMQKQLRQLQEKFYQVYDSTDSENDEDGDLSEDSMRSEILDARAQDSVGRSDNEMCELDPGQFIDRARALIREQEMAENKPKREGSNKERDHGPNSLQPEGKHLAETLKQELNTAMSQVVDTVVKVFSAKPSRQVPQVFPPLQIPQARFAVNGENHNFHTANQRLQCFGDVIIPNPLDTFGSVQMPSSTDQTEALPLVVRKNSSEQSASGPATGGHHQPLHQSPLSATAGFTTPSFRHPFPLPLMAYPFQSPLGAPSGSFSGKDRASPESLDLTRDTTSLRTKMSSHHLSHHPCSPAHPPSTAEGLSLSLIKSECGDLQDMSDISPYSGSAMQEGLSPNHLKKAKLMFFYTRYPSSNMLKTYFSDVKFNRCITSQLIKWFSNFREFYYIQMEKYARQAINDGVTSTEELSITRDCELYRALNMHYNKANDFEVPERFLEVAQITLREFFNAIIAGKDVDPSWKKAIYKVICKLDSEVPEIFKSPNCLQELLHE